European Patent Application EP 4 502 601 A1, published February 5, 2025. Title: 免疫学的検出方法及び免疫学的検出キット. Applicant: 積水メディカル株式会社. Application WO. The sequence listing filed with the application follows.

SEQUENCE LISTING (4 sequences)

SEQ ID NO: 1 - protein, 10 aa, Homo sapiens
QEEGQVEGQD

SEQ ID NO: 2 - protein, 13 aa, Homo sapiens
PDGSESPTDQETT

SEQ ID NO: 3 - protein, 11 aa, Homo sapiens
QEEGQVEGQDC

SEQ ID NO: 4 - protein, 14 aa, Homo sapiens
PDGSESPTDQETTC